European Patent Specification EP 3 881 849 B1, published April 30, 2025. Title: A COMPOSITION FOR TREATING AND PREVENTING DEGENERATIVE BRAIN DISEASES COMPRISING APTAMER. Applicant: Nexmos Co., Ltd. The sequence listing filed with the application follows.

SEQUENCE LISTING (1 sequence)

SEQ ID NO: 1 - DNA, 32 bp, Artificial Sequence
  aptamer
gtggaggcggtggccagtctcgcggtggcggc